European Patent Application EP 4 684 800 A1, published January 28, 2026. Title: Pharmaceutical composition for treating brain injuries. Applicant: 国立大学法人東京科学大学. Application EP 24775022.7, filed February 9, 2024. The sequence listing filed with the application follows.

SEQUENCE LISTING (18 sequences)

SEQ ID NO: 1 - DNA, 2782 bp, Mus musculus
  source 1..2782: mol_type = genomic DNA
  CDS 66..1637: protein_id = 2; translation = MEESHFNSNPYFWPSIPTVSGQIENTMFINKMKDQLLPEKGCGLAPPHYPTLLTVPASVSLSSGISMDTESKSEQLTPHSQASVTQNITVVPVPSTGLMTAGVSCSQRWRREGSQSRGPGLVITSPSGSLVTTASAAQTFPISAPMIVSALPPGSQALQVVPDLSKKVASTLTEEGGGGGGGGGTVAPPKPPRGRKKKRMLESGLPEMNDPYVLAPGDDDDHQKDGKTYRCRMCSLTFYSKSEMQIHSKSHTETKPHKCPHCSKTFANSSYLAQHIRIHSGAKPYSCNFCEKSFRQLSHLQQHTRIHTGDRPYKCAHPGCEKAFTQLSNLQSHRRQHNKDKPFKCHNCHRAYTDAASLEAHLSTHTVKHAKVYTCTICSRAYTSETYLMKHMRKHNPPDLQQQVQAAAAAAAVAQAQAQAQAQAQAQAQAQAQAQAQAQAQAQAQAQASQASQQQQQQQPPPQPPHFQSPGAAPQGGGGGDSNPNPPPQCSFDLTPYKPAEHHKDICLTVTTSTIQVEHLASS
aaagttcaggagccctggaaaggagaaggaataagacgacaggaggaagagagagagagggtagaatggaagagtctcacttcaattctaacccgtacttctggccttctatccccacagtctcagggcagattgaaaacactatgttcatcaacaagatgaaggatcagctgttgccagagaagggctgtggactggcgccacctcactatcccactttgctaactgtccctgcctcagtgtccctgtcctctggcatcagcatggacacagagtccaagtcagaacagctgaccccacacagtcaggcatctgttacccagaatatcacagtggttcctgtaccatctacaggactcatgactgcgggagtctcctgttctcagaggtggagaagagaagggagtcaatcaaggggtcctggtttggtaatcacatccccgtcaggctctcttgtgaccacagcctccgcagctcagactttccctatttcggctcccatgattgtctcagctcttcccccgggctcgcaagccctacaggtggtccctgacctctccaagaaggtagcgtcaaccctaactgaggaaggaggcggaggtggtggtggaggtggcactgtggctcctcctaaacctcctcggggccgcaagaagaagcggatgctggagtcagggcttcctgagatgaatgacccttacgtccttgcccctggggatgacgatgaccatcagaaagatggcaagacctacaggtgccggatgtgctccctgaccttctactccaagtcggagatgcagatccactccaagtcacacaccgagaccaagccccacaagtgcccgcactgctccaagaccttcgccaacagctcctacctggcccagcacatccggatccactcaggggccaagccctatagttgtaacttctgtgagaaatccttccgccagctctcacatctgcagcagcacacccgaatccacactggtgatagaccatacaaatgtgcacacccgggctgtgagaaggctttcacacaactctccaatctgcagtctcacagacggcagcacaacaaagataaacccttcaagtgccacaactgtcaccgagcatatacagacgcagcctctctcgaggctcacttatctacacacacagtgaaacacgccaaggtttatacctgcacaatctgcagtcgggcatatacatcagaaacataccttatgaaacatatgcgcaaacacaaccctcctgatcttcaacagcaagtgcaagcagcggcagcagcagcagcggtggcccaggcccaggcccaggctcaggcccaagctcaagcccaggcccaagctcaagcccaggcccaagctcaagcccaggcccaggcccaggcccaggcccaggcttcacaggcgtcacagcagcagcagcagcagcagccaccgccacaaccaccacacttccagtcccctggggcagctccccagggagggggtggtggggacagcaacccgaaccctccaccccagtgttcctttgacttgaccccctataagccggcagagcatcataaagacatctgcctcactgtcaccaccagcaccatccaggtggagcacctggccagctcttagagatccgtactgccatccatcggaacggggagaagtcctggtccctcctttgtcaactcttcttggtgggaaagttctcttcttccttgacaagtcctgtctccagctccttgggtctcaggcatggcttttcttcgcaagataaccatccttattctcagctgctcctgattggccaaggaatcctgagctgatagtgttatccaacagcccccatccaggcagagcttttaaaactggggcttggtgcttgagagaaggatccgctgggagctcacacatcttatccagtgtggggcgcttacctttctctctcttcatcctcaaagttgaggttgatggaagactagtggctggccctcccagataacagagaaggaagctctaaatgccaccagccttccgttctatgcttacctgtaaaagaacagattttgcacgtggcctgacccctgtgagccattttcttccccttccgtggtctcactttatattgggtgatgactatacctttttatttgtaagggggcaatagctgattcatggttgccaaggtgccagagattccccggtgaccaagggtggcttaagagtatgagttatttttccttaacagcctccttccttctctgccaaccaagggcctatatactcagtctcgctatcccagtccaaggagctctgggagctgtggtagctgtgttctctgcaataccattcggtcttttgcagagaagggagaattcagggcacacacaggactggacttagcctccctaggtgccacggtcagatgccggacatggatttatatataaatatatatatataaatatatatatatatacctgctcatcacggccatctttgttgtaaccatttctgtgtttataaatgcattatctctgagaattttcatattgatgttttatttttgtcttatttttttttctccaccttgtcctctggccatggcattttaattttcttttgacttttaatttttttaatcatgggagatttcagataaaataatcaggaattatacagttgttataaagcaatttaaaaatgaaaatcttatgtacaaactaaggggtgtttttagaccattgtatagaaataaattcatgtttaaggatgag

SEQ ID NO: 2 - protein, 523 aa, Mus musculus
MEESHFNSNPYFWPSIPTVSGQIENTMFINKMKDQLLPEKGCGLAPPHYPTLLTVPASVSLSSGISMDTESKSEQLTPHSQASVTQNITVVPVPSTGLMTAGVSCSQRWRREGSQSRGPGLVITSPSGSLVTTASAAQTFPISAPMIVSALPPGSQALQVVPDLSKKVASTLTEEGGGGGGGGGTVAPPKPPRGRKKKRMLESGLPEMNDPYVLAPGDDDDHQKDGKTYRCRMCSLTFYSKSEMQIHSKSHTETKPHKCPHCSKTFANSSYLAQHIRIHSGAKPYSCNFCEKSFRQLSHLQQHTRIHTGDRPYKCAHPGCEKAFTQLSNLQSHRRQHNKDKPFKCHNCHRAYTDAASLEAHLSTHTVKHAKVYTCTICSRAYTSETYLMKHMRKHNPPDLQQQVQAAAAAAAVAQAQAQAQAQAQAQAQAQAQAQAQAQAQAQAQAQASQASQQQQQQQPPPQPPHFQSPGAAPQGGGGGDSNPNPPPQCSFDLTPYKPAEHHKDICLTVTTSTIQVEHLASS

SEQ ID NO: 3 - DNA, 16 bp, synthetic oligonucleotide
  source 1..16: mol_type = unassigned DNA
ggatttctcacagaag

SEQ ID NO: 4 - DNA, 16 bp, synthetic oligonucleotide
  source 1..16: mol_type = unassigned DNA
gaaggatttctcacag

SEQ ID NO: 5 - DNA, 16 bp, synthetic oligonucleotide
  source 1..16: mol_type = unassigned DNA
ctcacagaagttacaa

SEQ ID NO: 6 - DNA, 16 bp, synthetic oligonucleotide
  source 1..16: mol_type = unassigned DNA
acatttgtatggtcta

SEQ ID NO: 7 - DNA, 16 bp, synthetic oligonucleotide
  source 1..16: mol_type = unassigned DNA
gcacatttgtatggtc

SEQ ID NO: 8 - DNA, 16 bp, synthetic oligonucleotide
  source 1..16: mol_type = unassigned DNA
tggagagttgtgtgaa

SEQ ID NO: 9 - DNA, 16 bp, synthetic oligonucleotide
  source 1..16: mol_type = unassigned DNA
gattggagagttgtgt

SEQ ID NO: 10 - DNA, 16 bp, synthetic oligonucleotide
  source 1..16: mol_type = unassigned DNA
agattggagagttgtg

SEQ ID NO: 11 - DNA, 16 bp, synthetic oligonucleotide
  source 1..16: mol_type = unassigned DNA
cagattggagagttgt

SEQ ID NO: 12 - DNA, 16 bp, synthetic oligonucleotide
  source 1..16: mol_type = unassigned DNA
gcacttgaagggttta

SEQ ID NO: 13 - DNA, 16 bp, synthetic oligonucleotide
  source 1..16: mol_type = unassigned DNA
tggcacttgaagggtt

SEQ ID NO: 14 - DNA, 16 bp, synthetic oligonucleotide
  source 1..16: mol_type = unassigned DNA
gtggcacttgaagggt

SEQ ID NO: 15 - RNA, 48 nt, synthetic oligonucleotide
  source 1..48: mol_type = other RNA
gctcagactttccctattttcaagagaaatagggaaagtctgagctgc

SEQ ID NO: 16 - DNA, 20 bp, synthetic oligonucleotide
  source 1..20: mol_type = other DNA
ctttttttgagaaaaaaaag

SEQ ID NO: 17 - RNA, 21 nt, synthetic oligonucleotide
  source 1..21: mol_type = other RNA
aatagggaaagtctgagctgc

SEQ ID NO: 18 - RNA, 21 nt, synthetic oligonucleotide
  source 1..21: mol_type = other RNA
gcagctcagactttccctatt